European Patent Application EP 4 606 900 A1, published August 27, 2025. Title: Modified RNA for the treatment of cfDNA-associated diseases. Applicant: ExploRNA THERAPEUTICS SP. Z O. O. The sequence listing filed with the application follows.

SEQUENCE LISTING (8 sequences)

SEQ ID NO: 1 - protein, 282 aa, Homo sapiens [sequence omitted]

SEQ ID NO: 2 - protein, 305 aa, Homo sapiens
MSRELAPLLLLLLSIHSALAMRICSFNVRSFGESKQEDKNAMDVIVKVIKRCDIILVMEIKDSNNRICPILMEKLNRNSRRGITYNYVISSRLGRNTYKEQYAFLYKEKLVSVKRSYHYHDYQDGDADVFSREPFVVWFQSPHTAVKDFVIIPLHTTPETSVKEIDELVEVYTDVKHRWKAENFIFMGDFNAGCSYVPKKAWKNIRLRTDPRFVWLIGDQEDTTVKKSTNCAYDRIVLRGQEIVSSVVPKSNSVFDFQKAYKLTEEEALDVSDHFPVEFKLQSSRAFTNSKKSVTLRKKTKSKRS

SEQ ID NO: 3 - DNA, 849 bp, synthetic construct
  source 1..849: mol_type = other DNA
atgaggggcatgaagctgctgggcgccctgctggccctggccgccctgctgcagggcgccgtgagcctgaagatcgccgccttcaacatccagaccttcggcgagaccaagatgagcaacgccaccctggtgagctacatcgtgcagatcctgagcaggtacgacatcgccctggtgcaggaggtgagggacagccacctgaccgccgtgggcaagctgctggacaacctgaaccaggacgcccccgacacctaccactacgtggtgagcgagcccctgggcaggaacagctacaaggagaggtacctgttcgtgtacaggcccgaccaggtgagcgccgtggacagctactactacgacgacggctgcgagccctgcggcaacgacaccttcaacagggagcccgccatcgtgaggttcttcagcaggttcaccgaggtgagggagttcgccatcgtgcccctgcacgccgcccccggcgacgccgtggccgagatcgacgccctgtacgacgtgtacctggacgtgcaggagaagtggggcctggaggacgtgatgctgatgggcgacttcaacgccggctgcagctacgtgaggcccagccagtggagcagcatcaggctgtggaccagccccaccttccagtggctgatccccgacagcgccgacaccaccgccacccccacccactgcgcctacgacaggatcgtggtggccggcatgctgctgaggggcgccgtggtgcccgacagcgccctgcccttcaacttccaggccgcctacggcctgagcgaccagctggcccaggccatcagcgaccactaccccgtggaggtgatgctgaagtga

SEQ ID NO: 4 - DNA, 918 bp, synthetic construct
  source 1..918: mol_type = other DNA
atgagcagggagctggcccccctgctgctgctgctgctgagcatccacagcgccctggccatgaggatctgcagcttcaacgtgaggagcttcggcgagagcaagcaggaggacaagaacgccatggacgtgatcgtgaaggtgatcaagaggtgcgacatcatcctggtgatggagatcaaggacagcaacaacaggatctgccccatcctgatggagaagctgaacaggaacagcaggaggggcatcacctacaactacgtgatcagcagcaggctgggcaggaacacctacaaggagcagtacgccttcctgtacaaggagaagctggtgagcgtgaagaggagctaccactaccacgactaccaggacggcgacgccgacgtgttcagcagggagcccttcgtggtgtggttccagagcccccacaccgccgtgaaggacttcgtgatcatccccctgcacaccacccccgagaccagcgtgaaggagatcgacgagctggtggaggtgtacaccgacgtgaagcacaggtggaaggccgagaacttcatcttcatgggcgacttcaacgccggctgcagctacgtgcccaagaaggcctggaagaacatcaggctgaggaccgaccccaggttcgtgtggctgatcggcgaccaggaggacaccaccgtgaagaagagcaccaactgcgcctacgacaggatcgtgctgaggggccaggagatcgtgagcagcgtggtgcccaagagcaacagcgtgttcgacttccagaaggcctacaagctgaccgaggaggaggccctggacgtgagcgaccacttccccgtggagttcaagctgcagagcagcagggccttcaccaacagcaagaagagcgtgaccctgaggaagaagaccaagagcaagaggagctga

SEQ ID NO: 5 - DNA, 1155 bp, synthetic construct
  source 1..1155: mol_type = other DNA
taatacgactcactatagggataatcataaaccctggcgcgctcgcggcccggcactcttctggtccccacagactcagagagaacccgccaccatgaggggcatgaagctgctgggcgccctgctggccctggccgccctgctgcagggcgccgtgagcctgaagatcgccgccttcaacatccagaccttcggcgagaccaagatgagcaacgccaccctggtgagctacatcgtgcagatcctgagcaggtacgacatcgccctggtgcaggaggtgagggacagccacctgaccgccgtgggcaagctgctggacaacctgaaccaggacgcccccgacacctaccactacgtggtgagcgagcccctgggcaggaacagctacaaggagaggtacctgttcgtgtacaggcccgaccaggtgagcgccgtggacagctactactacgacgacggctgcgagccctgcggcaacgacaccttcaacagggagcccgccatcgtgaggttcttcagcaggttcaccgaggtgagggagttcgccatcgtgcccctgcacgccgcccccggcgacgccgtggccgagatcgacgccctgtacgacgtgtacctggacgtgcaggagaagtggggcctggaggacgtgatgctgatgggcgacttcaacgccggctgcagctacgtgaggcccagccagtggagcagcatcaggctgtggaccagccccaccttccagtggctgatccccgacagcgccgacaccaccgccacccccacccactgcgcctacgacaggatcgtggtggccggcatgctgctgaggggcgccgtggtgcccgacagcgccctgcccttcaacttccaggccgcctacggcctgagcgaccagctggcccaggccatcagcgaccactaccccgtggaggtgatgctgaagtgaggatccgctggagcctcggtggcctagcttcttgccccttgggcctccccccagcccctcctccccttcctgcacccgtacccccgtggtctttgaataaagtctgagtgggcggcactagtaaaaaaaaaaaaaaaaaaaaaaaaaaaaaaaaaaaaaaaaaaaaaaaaaaaaaaaaaaaaaaaaaaaaaaaaaaaaaaaaaaaaaaaaaa

SEQ ID NO: 6 - DNA, 1159 bp, synthetic construct
  source 1..1159: mol_type = other DNA
taatacgactcactatagggataatacatttgcttctgacacaactgtgttcactagcaacctcaaacagacaccatgaggggcatgaagctgctgggcgccctgctggccctggccgccctgctgcagggcgccgtgagcctgaagatcgccgccttcaacatccagaccttcggcgagaccaagatgagcaacgccaccctggtgagctacatcgtgcagatcctgagcaggtacgacatcgccctggtgcaggaggtgagggacagccacctgaccgccgtgggcaagctgctggacaacctgaaccaggacgcccccgacacctaccactacgtggtgagcgagcccctgggcaggaacagctacaaggagaggtacctgttcgtgtacaggcccgaccaggtgagcgccgtggacagctactactacgacgacggctgcgagccctgcggcaacgacaccttcaacagggagcccgccatcgtgaggttcttcagcaggttcaccgaggtgagggagttcgccatcgtgcccctgcacgccgcccccggcgacgccgtggccgagatcgacgccctgtacgacgtgtacctggacgtgcaggagaagtggggcctggaggacgtgatgctgatgggcgacttcaacgccggctgcagctacgtgaggcccagccagtggagcagcatcaggctgtggaccagccccaccttccagtggctgatccccgacagcgccgacaccaccgccacccccacccactgcgcctacgacaggatcgtggtggccggcatgctgctgaggggcgccgtggtgcccgacagcgccctgcccttcaacttccaggccgcctacggcctgagcgaccagctggcccaggccatcagcgaccactaccccgtggaggtgatgctgaagtgaggatccagctcgctttcttgctgtccaatttctattaaaggttcctttgttccctaagtccaactactaaactgggggatattatgaagggccttgagcatttggattctgcctaataaaaaacatttattttcattgcactagtaaaaaaaaaaaaaaaaaaaaaaaaaaaaaaaaaaaaaaaaaaaaaaaaaaaaaaaaaaaaaaaaaaaaaaaaaaaaaaaaaaaaaaaaaa

SEQ ID NO: 7 - DNA, 1224 bp, synthetic construct
  source 1..1224: mol_type = other DNA
taatacgactcactatagggataatcataaaccctggcgcgctcgcggcccggcactcttctggtccccacagactcagagagaacccgccaccatgagcagggagctggcccccctgctgctgctgctgctgagcatccacagcgccctggccatgaggatctgcagcttcaacgtgaggagcttcggcgagagcaagcaggaggacaagaacgccatggacgtgatcgtgaaggtgatcaagaggtgcgacatcatcctggtgatggagatcaaggacagcaacaacaggatctgccccatcctgatggagaagctgaacaggaacagcaggaggggcatcacctacaactacgtgatcagcagcaggctgggcaggaacacctacaaggagcagtacgccttcctgtacaaggagaagctggtgagcgtgaagaggagctaccactaccacgactaccaggacggcgacgccgacgtgttcagcagggagcccttcgtggtgtggttccagagcccccacaccgccgtgaaggacttcgtgatcatccccctgcacaccacccccgagaccagcgtgaaggagatcgacgagctggtggaggtgtacaccgacgtgaagcacaggtggaaggccgagaacttcatcttcatgggcgacttcaacgccggctgcagctacgtgcccaagaaggcctggaagaacatcaggctgaggaccgaccccaggttcgtgtggctgatcggcgaccaggaggacaccaccgtgaagaagagcaccaactgcgcctacgacaggatcgtgctgaggggccaggagatcgtgagcagcgtggtgcccaagagcaacagcgtgttcgacttccagaaggcctacaagctgaccgaggaggaggccctggacgtgagcgaccacttccccgtggagttcaagctgcagagcagcagggccttcaccaacagcaagaagagcgtgaccctgaggaagaagaccaagagcaagaggagctgaggatccgctggagcctcggtggcctagcttcttgccccttgggcctccccccagcccctcctccccttcctgcacccgtacccccgtggtctttgaataaagtctgagtgggcggcactagtaaaaaaaaaaaaaaaaaaaaaaaaaaaaaaaaaaaaaaaaaaaaaaaaaaaaaaaaaaaaaaaaaaaaaaaaaaaaaaaaaaaaaaaaaa

SEQ ID NO: 8 - DNA, 1228 bp, synthetic construct
  source 1..1228: mol_type = other DNA
taatacgactcactatagggataatacatttgcttctgacacaactgtgttcactagcaacctcaaacagacaccatgagcagggagctggcccccctgctgctgctgctgctgagcatccacagcgccctggccatgaggatctgcagcttcaacgtgaggagcttcggcgagagcaagcaggaggacaagaacgccatggacgtgatcgtgaaggtgatcaagaggtgcgacatcatcctggtgatggagatcaaggacagcaacaacaggatctgccccatcctgatggagaagctgaacaggaacagcaggaggggcatcacctacaactacgtgatcagcagcaggctgggcaggaacacctacaaggagcagtacgccttcctgtacaaggagaagctggtgagcgtgaagaggagctaccactaccacgactaccaggacggcgacgccgacgtgttcagcagggagcccttcgtggtgtggttccagagcccccacaccgccgtgaaggacttcgtgatcatccccctgcacaccacccccgagaccagcgtgaaggagatcgacgagctggtggaggtgtacaccgacgtgaagcacaggtggaaggccgagaacttcatcttcatgggcgacttcaacgccggctgcagctacgtgcccaagaaggcctggaagaacatcaggctgaggaccgaccccaggttcgtgtggctgatcggcgaccaggaggacaccaccgtgaagaagagcaccaactgcgcctacgacaggatcgtgctgaggggccaggagatcgtgagcagcgtggtgcccaagagcaacagcgtgttcgacttccagaaggcctacaagctgaccgaggaggaggccctggacgtgagcgaccacttccccgtggagttcaagctgcagagcagcagggccttcaccaacagcaagaagagcgtgaccctgaggaagaagaccaagagcaagaggagctgaggatccagctcgctttcttgctgtccaatttctattaaaggttcctttgttccctaagtccaactactaaactgggggatattatgaagggccttgagcatttggattctgcctaataaaaaacatttattttcattgcactagtaaaaaaaaaaaaaaaaaaaaaaaaaaaaaaaaaaaaaaaaaaaaaaaaaaaaaaaaaaaaaaaaaaaaaaaaaaaaaaaaaaaaaaaaaa